European Patent Application EP 4 506 368 A1, published February 12, 2025. Title: Anti-human Tim-3 & anti-human CD39 bispecific antibody or antibody derivative and the use thereof. Applicant: ブライトパス・バイオ株式会社. Application JP. The sequence listing filed with the application follows.

SEQUENCE LISTING (126 sequences)

SEQ ID NO: 1 - protein, 5 aa, synthetic construct
  REGION 1..5: note = CDR1 of HC of anti-Tim3 Hu003_13_F20 antibody
SYYMS

SEQ ID NO: 2 - protein, 17 aa, synthetic construct
  REGION 1..17: note = CDR2 of HC of anti-Tim3 Hu003_13_F20 antibody
TISNSGGSTYYPDSVKD

SEQ ID NO: 3 - protein, 12 aa, synthetic construct
  REGION 1..12: note = CDR3 of HC of anti-Tim3 Hu003_13_F20 antibody
DPYYTNYVPMDY

SEQ ID NO: 4 - protein, 11 aa, synthetic construct
  REGION 1..11: note = CDR1 of LC of anti-Tim3 Hu003_13_F20 antibody
KASQYVDTYVA

SEQ ID NO: 5 - protein, 7 aa, synthetic construct
  REGION 1..7: note = CDR2 of LC of anti-Tim3 Hu003_13_F20 antibody
SASTRHT

SEQ ID NO: 6 - protein, 9 aa, synthetic construct
  REGION 1..9: note = CDR3 of LC of anti-Tim3 Hu003_13_F20 antibody
AQYSSSPLT

SEQ ID NO: 7 - protein, 121 aa, synthetic construct
  REGION 1..121: note = HC variable domain of anti-Tim3 Hu003_13_F20 antibody
QVQLQESGGGLVKPGGSLKLSCAASGFTFSSYYMSWVRQTPDKRLEWVATISNSGGSTYYPDSVKDRFTISRDNAKNTLYLQMSSLKSEDTAMYYCARDPYYTNYVPMDYWGQGTMVTVSS

SEQ ID NO: 8 - protein, 107 aa, synthetic construct
  REGION 1..107: note = LC variable domain of anti-Tim3 Hu003_13_F20 antibody
DIVMTQSPSFLSASVGDRVTITCKASQYVDTYVAWYQQRPGKAPKPLIYSASTRHTGVPSRFSGSGSGTEFTLTISSLQPEDFATYFCAQYSSSPLTFGGGTKLELK

SEQ ID NO: 9 - protein, 5 aa, synthetic construct
  REGION 1..5: note = CDR1 of HC of anti-Tim3 Hu149_83 antibody
DYYMD

SEQ ID NO: 10 - protein, 17 aa, synthetic construct
  REGION 1..17: note = CDR2 of HC of anti-Tim3 Hu149_83 antibody
YIYPNKGGTSYNQKFKG

SEQ ID NO: 11 - protein, 11 aa, synthetic construct
  REGION 1..11: note = CDR3 of HC of anti-Tim3 Hu149_83 antibody
SGYGNYYTMDY

SEQ ID NO: 12 - protein, 11 aa, synthetic construct
  REGION 1..11: note = CDR1 of LC of anti-Tim3 Hu149_83 antibody
KASQSVGNNVA

SEQ ID NO: 13 - protein, 7 aa, synthetic construct
  REGION 1..7: note = CDR2 of LC of anti-Tim3 Hu149_83 antibody
YASNRYT

SEQ ID NO: 14 - protein, 9 aa, synthetic construct
  REGION 1..9: note = CDR3 of LC of anti-Tim3 Hu149_83 antibody
QQHYSSPST

SEQ ID NO: 15 - protein, 120 aa, synthetic construct
  REGION 1..120: note = HC variable domain of anti-Tim3 Hu149_83 antibody
QVQLVQSGAEVKKPGASVKVSCKASGYTFTDYYMDWVRQAPGQGLEWLGYIYPNKGGTSYNQKFKGRVTMTTDKSTSTAYMELRSLRSDDTAVYYCARSGYGNYYTMDYWGQGTTVTVSS

SEQ ID NO: 16 - protein, 107 aa, synthetic construct
  REGION 1..107: note = LC variable domain of anti-Tim3 Hu149_83 antibody
DIVMTQSQKFMSTSVGDRVSITCKASQSVGNNVAWYQQKPGQSPKLLIYYASNRYTGVPDRFTGSGSGTDFTLTISNMQSEDLADYFCQQHYSSPSTFGGGTKLEIK

SEQ ID NO: 17 - protein, 5 aa, synthetic construct
  REGION 1..5: note = CDR1 of HC of anti-Tim3 Hu428_83 antibody
DYYMD

SEQ ID NO: 18 - protein, 17 aa, synthetic construct
  REGION 1..17: note = CDR2 of HC of anti-Tim3 Hu428_83 antibody
YIYPNKGGTSYNQKFKG

SEQ ID NO: 19 - protein, 11 aa, synthetic construct
  REGION 1..11: note = CDR3 of HC of anti-Tim3 Hu428_83 antibody
GGYYSYYSYDY

SEQ ID NO: 20 - protein, 11 aa, synthetic construct
  REGION 1..11: note = CDR1 of LC of anti-Tim3 Hu428_83 antibody
KASQSVGNNVA

SEQ ID NO: 21 - protein, 7 aa, synthetic construct
  REGION 1..7: note = CDR2 of LC of anti-Tim3 Hu428_83 antibody
YASNRYT

SEQ ID NO: 22 - protein, 9 aa, synthetic construct
  REGION 1..9: note = CDR3 of LC of anti-Tim3 Hu428_83 antibody
QQHYSSPYT

SEQ ID NO: 23 - protein, 120 aa, synthetic construct
  REGION 1..120: note = HC variable domain of anti-Tim3 Hu428_83 antibody
QVQLVQSGAEVKKPGASVKVSCKASGYTFTDYYMDWVRQAPGQGLEWLGYIYPNKGGTSYNQKFKGRVTMTTDKSTSTAYMELRSLRSDDTAVYYCARGGYYSYYSYDYWGQGTTVTVSS

SEQ ID NO: 24 - protein, 107 aa, synthetic construct
  REGION 1..107: note = LC variable domain of anti-Tim3 Hu428_83 antibody
DIVMTQSQKFMSTSVGDRVSITCKASQSVGNNVAWYQQKPGQSPKLLIYYASNRYTGVPDRFTGSGSGTDFTLTISNMQSEDLADYFCQQHYSSPYTFGGGTKLEIK

SEQ ID NO: 25 - protein, 5 aa, synthetic construct
  REGION 1..5: note = CDR1 of HC of anti-Tim3 Hu621_83 antibody
DYYMD

SEQ ID NO: 26 - protein, 17 aa, synthetic construct
  REGION 1..17: note = CDR2 of HC of anti-Tim3 Hu621_83 antibody
YIYPNKGGTSYNQKFKG

SEQ ID NO: 27 - protein, 11 aa, synthetic construct
  REGION 1..11: note = CDR3 of HC of anti-Tim3 Hu621_83 antibody
SGYKAYYAMDY

SEQ ID NO: 28 - protein, 11 aa, synthetic construct
  REGION 1..11: note = CDR1 of LC of anti-Tim3 Hu621_83 antibody
KASQSVGNNVA

SEQ ID NO: 29 - protein, 7 aa, synthetic construct
  REGION 1..7: note = CDR2 of LC of anti-Tim3 Hu621_83 antibody
YASNRYT

SEQ ID NO: 30 - protein, 9 aa, synthetic construct
  REGION 1..9: note = CDR3 of LC of anti-Tim3 Hu621_83 antibody
QQHYSSPYT

SEQ ID NO: 31 - protein, 120 aa, synthetic construct
  REGION 1..120: note = HC variable domain of anti-Tim3 Hu621_83 antibody
QVQLVQSGAEVKKPGASVKVSCKASGYTFTDYYMDWVRQAPGQGLEWLGYIYPNKGGTSYNQKFKGRVTMTTDKSTSTAYMELRSLRSDDTAVYYCARSGYKAYYAMDYWGQGTTVTVSS

SEQ ID NO: 32 - protein, 107 aa, synthetic construct; identical to SEQ ID NO: 24
  REGION 1..107: note = LC variable domain of anti-Tim3 Hu621_83 antibody

SEQ ID NO: 33 - protein, 5 aa, synthetic construct
  REGION 1..5: note = CDR1 of HC of anti-Tim3 072 antibody
SYYMS

SEQ ID NO: 34 - protein, 17 aa, synthetic construct
  REGION 1..17: note = CDR2 of HC of anti-Tim3 072 antibody
TISNSGGSTYYPDSVKD

SEQ ID NO: 35 - protein, 12 aa, synthetic construct
  REGION 1..12: note = CDR3 of HC of anti-Tim3 072 antibody
DPYYTNYVPMDY

SEQ ID NO: 36 - protein, 11 aa, synthetic construct
  REGION 1..11: note = CDR1 of LC of anti-Tim3 072 antibody
KASENVGTYVS

SEQ ID NO: 37 - protein, 7 aa, synthetic construct
  REGION 1..7: note = CDR2 of LC of anti-Tim3 072 antibody
GASNRYT

SEQ ID NO: 38 - protein, 9 aa, synthetic construct
  REGION 1..9: note = CDR3 of LC of anti-Tim3 072 antibody
GQSYSYPLT

SEQ ID NO: 39 - protein, 121 aa, synthetic construct; identical to SEQ ID NO: 7
  REGION 1..121: note = HC variable domain of anti-Tim3 072 antibody

SEQ ID NO: 40 - protein, 107 aa, synthetic construct
  REGION 1..107: note = LC variable domain of anti-Tim3 072 antibody
DIVMTQSPDSLAVSLGERVTLSCKASENVGTYVSWYQQKPRQPPKLLIYGASNRYTGVPDRFSGSGSGTDFTLTISSLQAEDVALYYCGQSYSYPLTFGQGTRLEIK

SEQ ID NO: 41 - protein, 8 aa, synthetic construct
  REGION 1..8: note = CDR1 of HC of anti-CD39 6-3hIG antibody
GFSIKDTY

SEQ ID NO: 42 - protein, 8 aa, synthetic construct
  REGION 1..8: note = CDR2 of HC of anti-CD39 6-3hIG antibody
IDPANVNT

SEQ ID NO: 43 - protein, 14 aa, synthetic construct
  REGION 1..14: note = CDR3 of HC of anti-CD39 6-3hIG antibody
ALYGYDDDAYYFDY

SEQ ID NO: 44 - protein, 10 aa, synthetic construct
  REGION 1..10: note = CDR1 of LC of anti-CD39 6-3hIG antibody
ESVDNYGISF

SEQ ID NO: 45 - skipped

SEQ ID NO: 46 - protein, 9 aa, synthetic construct
  REGION 1..9: note = CDR3 of LC of anti-CD39 6-3hIG antibody
QQSKEVPYT

SEQ ID NO: 47 - protein, 121 aa, synthetic construct
  REGION 1..121: note = HC variable domain of anti-CD39 6-3hIG antibody
QVQLVQSGAELVKPGASVKLSCKASGFSIKDTYVHWVKQAPGKGLEWIGKIDPANVNTKFDPKFQGRVTITADTSTNTAYLQLSSLRSEDTAVYYCALYGYDDDAYYFDYWGQGTLVTVSS

SEQ ID NO: 48 - protein, 111 aa, synthetic construct
  REGION 1..111: note = LC variable domain of anti-CD39 6-3hIG antibody
EIVLTQSPASLSVSPGERATISCRASESVDNYGISFMNWFQQKPGQAPKLLIYAASNQGSGVPARFSGSGSGTDFTLTISSLEPEDFAVYYCQQSKEVPYTFGQGTKLEIK

SEQ ID NO: 49 - protein, 8 aa, synthetic construct
  REGION 1..8: note = CDR1 of HC of anti-CD39 B23-7hIF antibody
GYSFTDYN

SEQ ID NO: 50 - protein, 8 aa, synthetic construct
  REGION 1..8: note = CDR2 of HC of anti-CD39 B23-7hIF antibody
IDPYSGGT

SEQ ID NO: 51 - protein, 14 aa, synthetic construct
  REGION 1..14: note = CDR3 of HC of anti-CD39 B23-7hIF antibody
GLYGYDDDANYFDD

SEQ ID NO: 52 - protein, 5 aa, synthetic construct
  REGION 1..5: note = CDR1 of LC of anti-CD39 B23-7hIF antibody
SSVSY

SEQ ID NO: 53 - skipped

SEQ ID NO: 54 - protein, 9 aa, synthetic construct
  REGION 1..9: note = CDR3 of LC of anti-CD39 B23-7hIF antibody
QQRSSYPLT

SEQ ID NO: 55 - protein, 121 aa, synthetic construct
  REGION 1..121: note = HC variable domain of anti-CD39 B23-7hIF antibody
EVQLVQSGGELVKPGASVKISCKVSGYSFTDYNLNWVRQAPGKGLEWVGNIDPYSGGTRYNQKFKGRFTITIDQSKNTAYMQLNSLRSEDTAVYYCGLYGYDDDANYFDDWGQGTLVTVSS

SEQ ID NO: 56 - protein, 106 aa, synthetic construct
  REGION 1..106: note = LC variable domain of anti-CD39 B23-7hIF antibody
EIVLTQSPASLSASPGERVTISCSASSSVSYMHWFQQKPGQAPKLWIYATSNLASGVPARFSGSGSGTDYTLTISSMEPEDFATYYCQQRSSYPLTFGQGTKVEIK

SEQ ID NO: 57 - protein, 5 aa, synthetic construct
  REGION 1..5: note = CDR1 of HC of anti-CD39 P4 antibody
NYGVH

SEQ ID NO: 58 - protein, 16 aa, synthetic construct
  REGION 1..16: note = CDR2 of HC of anti-CD39 P4 antibody
VILRRGSTDYNAAFMS

SEQ ID NO: 59 - protein, 11 aa, synthetic construct
  REGION 1..11: note = CDR3 of HC of anti-CD39 P4 antibody
TAVVAGDYFDY

SEQ ID NO: 60 - protein, 11 aa, synthetic construct
  REGION 1..11: note = CDR1 of LC of anti-CD39 P4 antibody
KASQNVGTNVA

SEQ ID NO: 61 - protein, 7 aa, synthetic construct
  REGION 1..7: note = CDR2 of LC of anti-CD39 P4 antibody
SASYRYS

SEQ ID NO: 62 - protein, 9 aa, synthetic construct
  REGION 1..9: note = CDR3 of LC of anti-CD39 P4 antibody
QQYNSYPLT

SEQ ID NO: 63 - protein, 111 aa, synthetic construct
  REGION 1..111: note = HC variable domain ofanti-CD39 P4 antibody
QVQLVESGGGVVQPGGSLRLSCVVSGFTLTNYGVHWVRQAPGKGLEWLAVILRRGSTDYNAAFMSRLAISKDNSKNTVYLELNSLRLDDTAVVAGDYFDYWGQGTTVTVSS

SEQ ID NO: 64 - protein, 111 aa, synthetic construct; identical to SEQ ID NO: 63
  REGION 1..107: note = LC variable domain ofanti-CD39 P4 antibody

SEQ ID NO: 65 - protein, 5 aa, synthetic construct
  REGION 1..5: note = CDR1 of HC of anti-CD39 T86 antibody
NYGMN

SEQ ID NO: 66 - protein, 17 aa, synthetic construct
  REGION 1..17: note = CDR2 of HC of anti-CD39 T86 antibody
WINTYTGEPTYADDFKG

SEQ ID NO: 67 - protein, 14 aa, synthetic construct
  REGION 1..14: note = CDR3 of HC of anti-CD39 T86 antibody
KGYYGYPNYYAMDY

SEQ ID NO: 68 - protein, 11 aa, synthetic construct
  REGION 1..11: note = CDR1 of LC of anti-CD39 T86 antibody
KASQNVGTAVA

SEQ ID NO: 69 - protein, 7 aa, synthetic construct
  REGION 1..7: note = CDR2 of LC of anti-CD39 T86 antibody
SASNRYT

SEQ ID NO: 70 - protein, 9 aa, synthetic construct
  REGION 1..9: note = CDR3 of LC of anti-CD39 T86 antibody
QQYSSYPIT

SEQ ID NO: 71 - protein, 123 aa, synthetic construct
  REGION 1..123: note = HC variable domain of anti-CD39 T86 antibody
QIQLVQSGPELKKPGETVKISCEASGYTFINYGMNWVKQAPGKGLKWMGWINTYTGEPTYADDFKGRFAFSLETSANTAYLQINNLKNEDTATYFCARKGYYGYPNYYAMDYWGQGTSVTVSS

SEQ ID NO: 72 - protein, 107 aa, synthetic construct
  REGION 1..107: note = LC variable domain of anti-CD39 T86 antibody
DIVMTQSQKFMSTSVGDRVSITCKASQNVGTAVAWYQQKPGQSPKLLIYSASNRYTGVPDRFTGSGSGTDFTLTISNMQSEDLADYFCQQYSSYPITFGTGTKLEIK

SEQ ID NO: 73 - protein, 5 aa, synthetic construct
  REGION 1..5: note = CDR1 of HC of anti-CD39 I67 antibody
SYGVH

SEQ ID NO: 74 - protein, 16 aa, synthetic construct
  REGION 1..16: note = CDR2 of HC of anti-CD39 I67 antibody
VIWRRGSTDYNAAFMS

SEQ ID NO: 75 - protein, 11 aa, synthetic construct
  REGION 1..11: note = CDR3 of HC of anti-CD39 I67 antibody
GISTATSWFAY

SEQ ID NO: 76 - protein, 11 aa, synthetic construct
  REGION 1..11: note = CDR1 of LC of anti-CD39 I67 antibody
KASQNVGTNVA

SEQ ID NO: 77 - protein, 7 aa, synthetic construct
  REGION 1..7: note = CDR2 of LC of anti-CD39 I67 antibody
SASYRYS

SEQ ID NO: 78 - protein, 9 aa, synthetic construct
  REGION 1..9: note = CDR3 of LC of anti-CD39 I67 antibody
QQYNSYPLT

SEQ ID NO: 79 - protein, 119 aa, synthetic construct
  REGION 1..119: note = HC variable domain of anti-CD39 I67 antibody
DVQLQESGPSLVQPSQSLSINCTVSGFSLSSYGVHWVRQSPGKGLEWLGVIWRRGSTDYNAAFMSRLSITKDNSKSQVFFKMNRLQADDTATYYCAKGISTATSWFAYWGQGTLVTVSA

SEQ ID NO: 80 - protein, 107 aa, synthetic construct
  REGION 1..107: note = LC variable domain of anti-CD39 I67 antibody
DIVMTQSHKFMSTSVGDRVSVTCKASQNVGTNVAWYQQKPGQSPKALIYSASYRYSGVPDRFTGSGSGTDFTLTISNVQSEDLAEYFCQQYNSYPLTFGAGTKLELK

SEQ ID NO: 81 - protein, 5 aa, synthetic construct
  REGION 1..5: note = CDR1 of HC of anti-CD39 Tre291 antibody
SYGVH

SEQ ID NO: 82 - protein, 16 aa, synthetic construct
  REGION 1..16: note = CDR2 of HC of anti-CD39 Tre291 antibody
VIWRRGSTDYNAAFMS

SEQ ID NO: 83 - protein, 8 aa, synthetic construct
  REGION 1..8: note = CDR3 of HC of anti-CD39 Tre291 antibody
VRGDAMDY

SEQ ID NO: 84 - protein, 11 aa, synthetic construct
  REGION 1..11: note = CDR1 of LC of anti-CD39 Tre291 antibody
KASQNVGTNVA

SEQ ID NO: 85 - protein, 7 aa, synthetic construct
  REGION 1..7: note = CDR2 of LC of anti-CD39 Tre291 antibody
SASYRYS

SEQ ID NO: 86 - protein, 9 aa, synthetic construct
  REGION 1..9: note = CDR3 of LC of anti-CD39 Tre291 antibody
QQYNSYPLT

SEQ ID NO: 87 - protein, 116 aa, synthetic construct
  REGION 1..116: note = HC variable domain of anti-CD39 Tre291 antibody
QVQLKQSGPGLVQPSQSLSITCTVSGFSLTSYGVHWVRQSPGKGLEWLGVIWRRGSTDYNAAFMSRLSITKDTSKSQVFFKMNSLQTDDTAIYYCAGVRGDAMDYWGQGTSVTVSS

SEQ ID NO: 88 - protein, 107 aa, synthetic construct
  REGION 1..107: note = LC variable domain of anti-CD39 Tre291 antibody
DIVMTQSHKSMSTSVGDRVSVTCKASQNVGTNVAWYQQKPGQSPKALIYSASYRYSGVPDRFTGSGSGTDFTLTISNVQSEDLAEYFCQQYNSYPLTFGGGTKLEIK

SEQ ID NO: 89 - protein, 5 aa, synthetic construct
  REGION 1..5: note = CDR1 of HC of anti-CD39 mAnE67 antibody
DYGMH

SEQ ID NO: 90 - protein, 17 aa, synthetic construct
  REGION 1..17: note = CDR2 of HC of anti-CD39 mAnE67 antibody
YISSGSSIIYYADTVKG

SEQ ID NO: 91 - protein, 9 aa, synthetic construct
  REGION 1..9: note = CDR3 of HC of anti-CD39 mAnE67 antibody
KDYPYAMDY

SEQ ID NO: 92 - protein, 11 aa, synthetic construct
  REGION 1..11: note = CDR1 of LC of anti-CD39 mAnE67 antibody
KASQNVGTNVA

SEQ ID NO: 93 - protein, 7 aa, synthetic construct
  REGION 1..7: note = CDR2 of LC of anti-CD39 mAnE67 antibody
WASNRFT

SEQ ID NO: 94 - protein, 9 aa, synthetic construct
  REGION 1..9: note = CDR3 of LC of anti-CD39 mAnE67 antibody
QQYSSSPYT

SEQ ID NO: 95 - protein, 118 aa, synthetic construct
  REGION 1..118: note = HC variable domain of anti-CD39 mAnE67 antibody
EVQLVESGGGLVKPGGSRKLSCAASGFTFSDYGMHWVRQAPEKGLEWVAYISSGSSIIYYADTVKGRFTISRDNAKNTLFLQMTGLRSEDTAMYYCARKDYPYAMDYWGQGTSLAVSS

SEQ ID NO: 96 - protein, 107 aa, synthetic construct
  REGION 1..107: note = LC variable domain of anti-CD39 mAnE67 antibody
SIVMTQTPKFMSTSVGDRVSVTCKASQNVGTNVAWYQQKPGQSPKALIYWASNRFTGVPDRFTGSGSGTDFTLTISNVQSEDLADYFCQQYSSSPYTFGSGTKLEIK

SEQ ID NO: 97 - protein, 121 aa, synthetic construct
  REGION 1..121: note = HC variable domain of anti-CD39 6-3hIB antibody
QVQLLQSGAEVKKPGATVKISCKVSGFSIKDTYVHWVRQPPEQGLEWIGKIDPANVNTKFDPKFQGRLTITADTSKNTAYLELSSLRSEDTAVYYCALYGYDDDAYYFDYWGQGTLLTVSS

SEQ ID NO: 98 - protein, 111 aa, synthetic construct
  REGION 1..111: note = LC variable domain of anti-CD39 6-3hIB antibody
DIVLTQSPATLALSVGQRATLSCRASESVDNYGISFMNWFQQKPGQPPRLLIYAASNQGSGIPARFSGSGSGTDFTLTINPLESEDFAVYYCQQSKEVPYTFGPGTKLEIK

SEQ ID NO: 99 - protein, 121 aa, synthetic construct
  REGION 1..121: note = HC variable domain of anti-CD39 6-3hIF antibody
QVQLVQSGAELVKPGASVKLSCAASGFSIKDTYVHWVRQAPGKGLEWVGKIDPANVNTKFDPKFQGRFTITADTSKNTAYLQLSSLRSEDTAVYYCALYGYDDDAYYFDYWGQGTLVTVSS

SEQ ID NO: 100 - protein, 111 aa, synthetic construct
  REGION 1..111: note = LC variable domain of anti-CD39 6-3hIF antibody
DIVLTQSPASLSVSPGDRATISCRASESVDNYGISFMNWFQQKPGQAPKLLIYAASNQGSGVPARFSGSGSGTDFTLTISSLEPEDFAVYYCQQSKEVPYTFGQGTKLEIK

SEQ ID NO: 101 - protein, 121 aa, synthetic construct
  REGION 1..121: note = HC variable domain of anti-CD39 6-3hCB antibody
QVQLLQSGAEVVKPGATVKISCKVSGFSIKDTYVHWVRQPPGQGLEWIGKIDPANVNTKFDPKFQGRFTITADTSINTAYLELSSLTSEDTAVYYCALYGYDDDAYYFDYWGQGTLVTVSS

SEQ ID NO: 102 - protein, 111 aa, synthetic construct
  REGION 1..111: note = LC variable domain of anti-CD39 6-3hCB antibody
NIVLTQSPATLSLSLGQRATISCRASESVDNYGISFMNWFQQKPGQPPQLLIYAASNQGSGIPARFSGSGSGTDFTLNINPLESEDFAVYYCQQSKEVPYTFGPGTKLEIK

SEQ ID NO: 103 - protein, 121 aa, synthetic construct
  REGION 1..121: note = HC variable domain of anti-CD39 6-3hHB antibody
QVQLQQSGAELKKPGASVKISCKVSGFSIKDTYVHWVRQPPGKGLEWIGKIDPANVNTKFDPKFQGRFTITADTSTDTAYLELSSLRSEDTAVYYCALYGYDDDAYYFDYWGQGTMLTVSS

SEQ ID NO: 104 - protein, 111 aa, synthetic construct
  REGION 1..111: note = LC variable domain of anti-CD39 6-3hHB antibody
DIVLTQSPATLSLSLGQRATLSCRASESVDNYGISFMNWFQQKPGQPPRLLIYAASNQGSGIPARFSGSGSGTDFTLNITPLESEDFAVYYCQQSKEVPYTFGPGTKLELK

SEQ ID NO: 105 - protein, 121 aa, synthetic construct
  REGION 1..121: note = HC variable domain of anti-CD39 6-3hKB antibody
QVQLLQSGAEVVKPGATVKISCKVSGFSIKDTYVHWVRQRPERGLEWIGKIDPANVNTKFDPKFQGRLTITADTSTDTAYLELSSLRSEDTAVYYCALYGYDDDAYYFDYWGQGTLLTVSS

SEQ ID NO: 106 - protein, 111 aa, synthetic construct
  REGION 1..111: note = LC variable domain of anti-CD39 6-3hKB antibody
DIVLTQSPATLSLSPGQRATISCRASESVDNYGISFMNWFQQKPGQPPRLLIYAASNQGSGIPARFSGSGSGTDFTLNIHPLESEDFAVYYCQQSKEVPYTFGPGTKLEIK

SEQ ID NO: 107 - protein, 121 aa, synthetic construct
  REGION 1..121: note = HC variable domain of anti-CD39 B23-7hIB antibody
EVQLLQSGPEVVKPGATVKISCKVSGYSFTDYNLNWVKQPPGKNLEWIGNIDPYSGGTRYNQKFKGRFTITIDQSINTAYMELRSLTSEDTAVYYCGLYGYDDDANYFDDWGQGTMLTVSS

SEQ ID NO: 108 - protein, 106 aa, synthetic construct
  REGION 1..106: note = LC variable domain of anti-CD39 B23-7hIB antibody
EIVLTQSPAILSPSPGERVTLNCSASSSVSYMHWFQQKPGQAPRLWIYATSNLASGIPARFSGSGSGTEYTLTISRMESEDFAVYYCQQRSSYPLTFGQGTKLEIK

SEQ ID NO: 109 - protein, 121 aa, synthetic construct
  REGION 1..121: note = HC variable domain of anti-CD39 B23-7hIG antibody
EVQLVQSGAELKKPGASVKISCKVSGYSFTDYNLNWVKQAPGKGLEWIGNIDPYSGGTRYNQKFKGRVTITIDQSTSTAYMELSSLRSEDTAVYYCGLYGYDDDANYFDDWGQGTLVTVSS

SEQ ID NO: 110 - protein, 106 aa, synthetic construct
  REGION 1..106: note = LC variable domain of anti-CD39 B23-7hIG antibody
EIVLTQSPATLSLSPGERATISCSASSSVSYMHWFQQKPGQAPKLWIYATSNLASGVPARFSGSGSGTDYTLTISSMEPEDFAVYYCQQRSSYPLTFGGGTKVEIK

SEQ ID NO: 111 - protein, 121 aa, synthetic construct
  REGION 1..121: note = HC variable domain of anti-CD39 B23-7hCB antibody
EVQLVQSGPEVKKPGATVKISCKVSGYSFTDYNLNWVKQPPGKNLEWIGNIDPYSGGTRYNQKFKGRFTITIDQSINTAYMHLRSLRSEDTAVYYCGLYGYDDDANYFDDWGQGTMLTVSS

SEQ ID NO: 112 - protein, 106 aa, synthetic construct
  REGION 1..106: note = LC variable domain of anti-CD39 B23-7hCB antibody
EIVLTQSPATLSPSPGERVTINCSASSSVSYMHWFQQKPGTPPRLWIYATSNLASGIPARFSGSGSGTEYTLTISSMESEDFAVYYCQQRSSYPLTFGPGTKVEIK

SEQ ID NO: 113 - protein, 121 aa, synthetic construct
  REGION 1..118: note = HC variable domain of anti-CD39 B23-7hHB antibody
EVQLLQSGPEVVKPGATVKISCKVSGYSFTDYNLNWVRQYPGKNLEWVGNIDPYSGGTRYNQKFKGRFTITIDQSKNTAYMELRSLTSEDTAVYYCGLYGYDDDANYFDDWGQGTMLTVSS

SEQ ID NO: 114 - protein, 106 aa, synthetic construct
  REGION 1..106: note = LC variable domain of anti-CD39 B23-7hHB antibody
EIVLTQSPAILSLSPGERVTITCSASSSVSYMHWFQQKPGQAPRLWIYATSNLASGIPARFSGSGSGTEYTLTISSMESEDFAVYYCQQRSSYPLTFGQGTKLEIK

SEQ ID NO: 115 - protein, 121 aa, synthetic construct
  REGION 1..118: note = HC variable domain of anti-CD39 B23-7hKB antibody
EVQLLQSGAEVVKPGATVKISCKVSGYSFTDYNLNWVKQPNGKNLEWIGNIDPYSGGTRYNQKFKGRFTITIDQSINTAYMQLNSLRSEDTAVYYCGLYGYDDDANYFDDWGQGTLLTVSS

SEQ ID NO: 116 - protein, 106 aa, synthetic construct
  REGION 1..106: note = LC variable domain of anti-CD39 B23-7hKB antibody
EIVLTQSPAILSPSPGERVTLTCSASSSVSYMHWFQQKPGKPPRLWIYATSNLASGIPARFSGSGSGTEYTLTISRMESEDFAVYYCQQRSSYPLTFGQGTKLEIK

SEQ ID NO: 117 - DNA, 1386 bp, synthetic construct
  misc_feature 1..1386: note = Fusion of TIM-3 & Fc antigen
  source 1..1386: mol_type = other DNA
  CDS 1..1386
atggagacagacacactcctgctatgggtactgctgctctgggttccaggttccactggtgactcagaagtggaatacagagcggaggtcggtcagaatgcctatctgccctgcttctacaccccagccgccccagggaacctcgtgcccgtctgctggggcaaaggagcctgtcctgtgtttgaatgtggcaacgtggtgctcaggactgatgaaagggatgtgaattattggacatccagatactggctaaatggggatttccgcaaaggagatgtgtccctgaccatagagaatgtgactctagcagacagtgggatctactgctgccggatccaaatcccaggcataatgaatgatgaaaaatttaacctgaagttggtcatcaaaccagccaaggtcacccctgcaccgactctgcagagagacttcactgcagcctttccaaggatgcttaccaccaggggacatggcccagcagagacacagacactggggagcctccctgatataaatctaacacaaatatccacattggccaatgagttacgggactctagattggccaatgacttacgggactctggagcaaccatcagaatcgagggcagaatggatcccaaatcttgtgacaaaactcacacatgcccaccgtgcccagcacctgaactcctggggggaccgtcagtcttcctcttccccccaaaacccaaggacaccctcatgatctcccggacccctgaggtcacatgcgtggtggtggacgtgagccacgaagaccctgaggtcaagttcaactggtacgtggacggcgtggaggtgcataatgccaagacaaagccgcgggaggagcagtacaacagcacgtaccgtgtggtcagcgtcctcaccgtcctgcaccaggactggctgaatggcaaggagtacaagtgcaaggtctccaacaaagccctcccagcccccatcgagaaaaccatctccaaagccaaagggcagccccgagaaccacaggtgtacaccctgcccccatcccgggaggagatgaccaagaaccaggtcagcctgacctgcctggtcaaaggcttctatcccagcgacatcgccgtggagtgggagagcaatgggcagccggagaacaactacaagaccacgcctcccgtgctggactccgacggctccttcttcctctacagcaagctcaccgtggacaagagcaggtggcagcaggggaacgtcttctcatgctccgtgatgcatgaggctctgcacaaccactacacgcagaagagcctctccctgtctccgggtaaaggtggcggtctgaacgacatcttcgaggctcagaaaatcgaatggcacgaacatcatcatcatcatcattgatag

SEQ ID NO: 118 - protein, 460 aa, synthetic construct
  REGION 1..460: note = Synthetic Construct
METDTLLLWVLLLWVPGSTGDSEVEYRAEVGQNAYLPCFYTPAAPGNLVPVCWGKGACPVFECGNVVLRTDERDVNYWTSRYWLNGDFRKGDVSLTIENVTLADSGIYCCRIQIPGIMNDEKFNLKLVIKPAKVTPAPTLQRDFTAAFPRMLTTRGHGPAETQTLGSLPDINLTQISTLANELRDSRLANDLRDSGATIRIEGRMDPKSCDKTHTCPPCPAPELLGGPSVFLFPPKPKDTLMISRTPEVTCVVVDVSHEDPEVKFNWYVDGVEVHNAKTKPREEQYNSTYRVVSVLTVLHQDWLNGKEYKCKVSNKALPAPIEKTISKAKGQPREPQVYTLPPSREEMTKNQVSLTCLVKGFYPSDIAVEWESNGQPENNYKTTPPVLDSDGSFFLYSKLTVDKSRWQQGNVFSCSVMHEALHNHYTQKSLSLSPGKGGGLNDIFEAQKIEWHEHHHHHH

SEQ ID NO: 119 - protein, 111 aa, synthetic construct
EVQLVESGGALVQPGRSLRLSCAVSGFTLSNYGVHWVRQAPGKGLEWVAVILRRGSTDYNAAFMSRFTISKDNSKNTVYLQMNSLRADDTAVVAGDYFDYWGQGTTVTVSS

SEQ ID NO: 120 - protein, 107 aa, synthetic construct
DIVMTQSQKFMSTSVGDRVSITCKASQNVGTNVAWYQQKPGQSPKLLIYSASYRYSGVPDRFTGSGSGTDFTLTISNMQSEDLADYFCQQYNSYPLTFGGGTKLEIK

SEQ ID NO: 121 - protein, 111 aa, synthetic construct
QVQLVESGGGVVQPGGSLRLSCVVSGFSLTNYGVHWVRQAPGKGLEWLGVILRRGSTDYNAAFMSRLAISKDNSKNTVYLELNSLRLDDTAVVAGDYFDYWGQGTTVTVSS

SEQ ID NO: 122 - protein, 107 aa, synthetic construct; identical to SEQ ID NO: 120

SEQ ID NO: 123 - protein, 111 aa, synthetic construct
QVQLLESGPELVKPSATLSITCTVSGFSLTNYGVHWIRQAPGKGLEWLGVILRRGSTDYNAAFMSRFTISKDNSKNQVYFKLRSVTAEDTAVVAGDYFDYWGQGTMVTVSS

SEQ ID NO: 124 - protein, 107 aa, synthetic construct
DIQMTQSHSTLSLSVGDRVTITCKASQNVGTNVAWYQQKPGQPPKALIYSASYRYSGVPSRFSGSGSGTDFTLTISSVQAEDVAVYYCQQYNSYPLTFGPGTKLEIK

SEQ ID NO: 125 - protein, 121 aa, synthetic construct; identical to SEQ ID NO: 7

SEQ ID NO: 126 - protein, 107 aa, synthetic construct
NIVMTQSPDSLAVSLGERATINCKASENVGTYVSWYQQKPGQPPKLLIYGASNRYTGVPDRFSGSGSGTDFTLTISSLQAEDVAVYYCGQSYSYPLTFGQGTKLEIK